European Patent Application EP 4 276 196 A1, published November 15, 2023. Title: Decoy-oligonucleotides in nucleic acid detection methods. Applicant: Philipps-Universität Marburg. The sequence listing filed with the application follows.

SEQUENCE LISTING (12 sequences)

SEQ ID NO: 1 - DNA, 256 bp, Artificial Sequence
  synthetic spike fragment
gttggtggtaattataattacctgtatagattgtttaggaagtctaatctcaaaccttttgagagagatatttcaactgaaatctatcaggccggtagcacaccttgtaatggtgttgaaggttttaattgttactttcctttacaatcatatggtttccaacccactaatggtgttggttaccaaccatacagagtagtagtactttcttttgaacttctacatgcaccagcaactgtttgtggacctaaaaagt

SEQ ID NO: 2 - DNA, 32 bp, Artificial Sequence
  spike_forward primer
aaatctatcaggccggtagcacaccttgtaat

SEQ ID NO: 3 - DNA, 32 bp, Artificial Sequence
  spike_reverse
aagaaagtactactactctgtatggttggtaa

SEQ ID NO: 4 - DNA, 48 bp, Artificial Sequence
  spikeP1-Targetsequenz
aaggttttaattgttactttcctttacaatcatatggtttccaaccca

SEQ ID NO: 5 - DNA, 48 bp, Artificial Sequence
  spikeP1-Sequenz
  misc_feature 33: /function="n= abasic position"
aaggttttaattgttactttcctttacaatcanatggtttccaaccca

SEQ ID NO: 6 - DNA, 30 bp, Artificial Sequence
  decoy2
ctattggtttccaacccactaatggtgttg

SEQ ID NO: 7 - DNA, 27 bp, Artificial Sequence
  decoy2c
ttggtttccaacccactaatggtgttg

SEQ ID NO: 8 - DNA, 27 bp, Artificial Sequence
  decoy2d
atggtttccaacccactaatggtgttg

SEQ ID NO: 9 - DNA, 26 bp, Artificial Sequence
  decoy2e
tggtttccaacccactaatggtgttg

SEQ ID NO: 10 - DNA, 25 bp, Artificial Sequence
  decoy2f
ggtttccaacccactaatggtgttg

SEQ ID NO: 11 - DNA, 30 bp, Artificial Sequence
  decoy1
ttcctttacaatctattggtttccaaccca

SEQ ID NO: 12 - DNA, 30 bp, Artificial Sequence
  decoy3
catatggtttccaacccactaatggtgttg